European Patent Specification EP 3 027 617 B1, published February 18, 2026. Title: METHODS AND COMPOUNDS USEFUL IN CONDITIONS RELATED TO REPEAT EXPANSION. Applicant: Ionis Pharmaceuticals, Inc. Board of Regents of the University of Texas System. Application 14832900.6. The sequence listing filed with the application follows.

SEQUENCE LISTING (45 sequences)

SEQ ID NO: 1 - DNA, 20 bp, Artificial Sequence
  Primer
ggaaatatggatgacagtgg

SEQ ID NO: 2 - DNA, 20 bp, Artificial Sequence
  Primer
atcctgagcctctgatactc

SEQ ID NO: 3 - DNA, 25 bp, Artificial Sequence
  Primer
gatgaggaagcagatctccgcaggg

SEQ ID NO: 4 - DNA, 26 bp, Artificial Sequence
  Primer
aagacatggtcacagctgcctgaagc

SEQ ID NO: 5 - DNA, 28 bp, Artificial Sequence
  Primer
gatttgcagagggctctggcactaagtc

SEQ ID NO: 6 - DNA, 33 bp, Artificial sequence
  Primer
agcatgtcttcttcactcatagcatcacttttc

SEQ ID NO: 7 - DNA, 21 bp, Artificial sequence
  Synthetic Oligonucleotide
  misc_feature (2)..(21): Bases at these positions are RNA
tcuacugcugcugcugcugaa

SEQ ID NO: 8 - DNA, 21 bp, Artificial sequence
  Synthetic Oligonucleotide
  misc_feature (2)..(21): Bases at these positions are RNA
tcugaugcugcugcugcugaa

SEQ ID NO: 9 - DNA, 21 bp, Artificial sequence
  Synthetic Oligonucleotide
  misc_feature (2)..(21): Bases at these positions are RNA
tcugcagcugcugcugcugaa

SEQ ID NO: 10 - DNA, 21 bp, Artificial sequence
  Synthetic Oligonucleotide
  misc_feature (2)..(21): Bases at these positions are RNA
tcugcuacugcugcugcugaa

SEQ ID NO: 11 - DNA, 21 bp, Artificial sequence
  Synthetic Oligonucleotide
  misc_feature (2)..(21): Bases at these positions are RNA
tcugcugaugcugcugcugaa

SEQ ID NO: 12 - DNA, 21 bp, Artificial sequence
  Synthetic Oligonucleotide
  misc_feature (2)..(21): Bases at these positions are RNA
tcugcugcagcugcugcugaa

SEQ ID NO: 13 - DNA, 21 bp, Artificial sequence
  Synthetic Oligonucleotide
  misc_feature (2)..(21): Bases at these positions are RNA
tcugcugcuacugcugcugaa

SEQ ID NO: 14 - DNA, 21 bp, Artificial sequence
  Synthetic Oligonucleotide
  misc_feature (2)..(21): Bases at these positions are RNA
tcugcugcuucugcugcugaa

SEQ ID NO: 15 - DNA, 21 bp, Artificial sequence
  Synthetic Oligonucleotide
  misc_feature (2)..(21): Bases at these positions are RNA
tcugcugcugaugcugcugaa

SEQ ID NO: 16 - DNA, 21 bp, Artificial sequence
  Synthetic Oligonucleotide
  misc_feature (2)..(21): Bases at these positions are RNA
tcugcugcugcagcugcugaa

SEQ ID NO: 17 - DNA, 21 bp, Artificial sequence
  Synthetic Oligonucleotide
  misc_feature (2)..(21): Bases at these positions are RNA
tcugcugcugcuacugcugaa

SEQ ID NO: 18 - DNA, 21 bp, Artificial sequence
  Synthetic Oligonucleotide
  misc_feature (2)..(21): Bases at these positions are RNA
tcugcugcugcugcuacugaa

SEQ ID NO: 19 - DNA, 21 bp, Artificial sequence
  Synthetic Oligonucleotide
  misc_feature (2)..(21): Bases at these positions are RNA
tcugcugcaacugcugcugaa

SEQ ID NO: 20 - DNA, 21 bp, Artificial sequence
  Synthetic Oligonucleotide
  misc_feature (2)..(21): Bases at these positions are RNA
tcugcugcaaaugcugcugaa

SEQ ID NO: 21 - DNA, 21 bp, Artificial sequence
  Synthetic Oligonucleotide
  misc_feature (2)..(21): Bases at these positions are RNA
tcugcugaaaaugcugcugaa

SEQ ID NO: 22 - DNA, 21 bp, Artificial sequence
  Synthetic Oligonucleotide
  misc_feature (2)..(21): Bases at these positions are RNA
tcuacugcuacugcuacugaa

SEQ ID NO: 23 - DNA, 21 bp, Artificial sequence
  Synthetic Oligonucleotide
  misc_feature (2)..(21): Bases at these positions are RNA
tcagcuguugcuacuguugaa

SEQ ID NO: 24 - DNA, 21 bp, Artificial sequence
  Synthetic Oligonucleotide
  misc_feature (2)..(21): Bases at these positions are RNA
tgcugcugcugcugcugcuaa

SEQ ID NO: 25 - DNA, 20 bp, Artificial sequence
  Synthetic Oligonucleotide
  misc_feature (2)..(20): Bases at these positions are RNA
tcugcugcagcugcugcuaa

SEQ ID NO: 26 - DNA, 19 bp, Artificial sequence
  Synthetic Oligonucleotide
  misc_feature (2)..(19): Bases at these positions are RNA
tcugcugcagcugcugcaa

SEQ ID NO: 27 - DNA, 18 bp, Artificial sequence
  Synthetic Oligonucleotide
  misc_feature (2)..(18): Bases at these positions are RNA
tcugcugcagcugcugaa

SEQ ID NO: 28 - DNA, 17 bp, Artificial sequence
  Synthetic Oligonucleotide
  misc_feature (2)..(17): Bases at these positions are RNA
tcugcugcagcugcuaa

SEQ ID NO: 29 - DNA, 16 bp, Artificial sequence
  Synthetic Oligonucleotide
  misc_feature (2)..(16): Bases at these positions are RNA
tcugcugcagcugcaa

SEQ ID NO: 30 - DNA, 15 bp, Artificial sequence
  Synthetic Oligonucleotide
  misc_feature (2)..(15): Bases at these positions are RNA
tcugcugcagcugaa

SEQ ID NO: 31 - DNA, 21 bp, Artificial sequence
  Synthetic Oligonucleotide
  misc_feature (2)..(21): Bases at these positions are RNA
tcugcugcagaugcugcugaa

SEQ ID NO: 32 - DNA, 21 bp, Artificial sequence
  Synthetic Oligonucleotide
  misc_feature (2)..(21): Bases at these positions are RNA
tcugcugcagcagcugcugaa

SEQ ID NO: 33 - DNA, 21 bp, Artificial sequence
  Synthetic Oligonucleotide
  misc_feature (2)..(21): Bases at these positions are RNA
tcugcugcagcuacugcugaa

SEQ ID NO: 34 - DNA, 21 bp, Artificial sequence
  Synthetic Oligonucleotide
  misc_feature (2)..(21): Bases at these positions are RNA
tcugcugcagcugaugcugaa

SEQ ID NO: 35 - DNA, 21 bp, Artificial sequence
  Synthetic Oligonucleotide
  misc_feature (2)..(21): Bases at these positions are RNA
tcugcugcagcugcagcugaa

SEQ ID NO: 36 - DNA, 21 bp, Artificial sequence
  Synthetic Oligonucleotide
  misc_feature (2)..(21): Bases at these positions are RNA
tcugcugcagcugcuccugaa

SEQ ID NO: 37 - DNA, 21 bp, Artificial sequence
  Synthetic Oligonucleotide
  misc_feature (2)..(21): Bases at these positions are RNA
tcugcugcagcugcugaugaa

SEQ ID NO: 38 - DNA, 21 bp, Artificial sequence
  Synthetic Oligonucleotide
  misc_feature (2)..(21): Bases at these positions are RNA
tcugcugcagcugcugcagaa

SEQ ID NO: 39 - DNA, 21 bp, Artificial sequence
  Synthetic Oligonucleotide
  misc_feature (2)..(21): Bases at these positions are RNA
tcugcugcagcugccgcugaa

SEQ ID NO: 40 - DNA, 21 bp, Artificial sequence
  Synthetic Oligonucleotide
  misc_feature (2)..(21): Bases at these positions are RNA
tcugcugcagcugcugccgaa

SEQ ID NO: 41 - RNA, 19 nt, Artificial sequence
  Synthetic Oligonucleotide
gcugcugcugcugcugcug

SEQ ID NO: 42 - DNA, 19 bp, Artificial sequence
  Synthetic Oligonucleotide
gctgctgctgctgctgctg

SEQ ID NO: 43 - DNA, 19 bp, Artificial sequence
  Synthetic Oligonucleotide
ctgctgctgctgctgctgc

SEQ ID NO: 44 - DNA, 19 bp, Artificial sequence
  Synthetic Oligonucleotide
tgctgctgctgctgctgct

SEQ ID NO: 45 - DNA, 19 bp, Artificial sequence
  Synthetic Oligonucleotide
tgctgctgctgctgctggc